European Patent Application EP 4 810 062 A1, published September 23, 2026. Title: 配体-药物偶联物、偶联连接子及其用途. Applicant: 海南先声再明医药股份有限公司. The sequence listing filed with the application follows.

SEQUENCE LISTING (22 sequences)

SEQ ID NO: 1 - protein, 120 aa, synthetic construct [sequence omitted]

SEQ ID NO: 2 - protein, 107 aa, synthetic construct [sequence omitted]

SEQ ID NO: 3 - protein, 330 aa, synthetic construct
ASTKGPSVFPLAPSSKSTSGGTAALGCLVKDYFPEPVTVSWNSGALTSGVHTFPAVLQSSGLYSLSSVVTVPSSSLGTQTYICNVNHKPSNTKVDKKVEPKSCDKTHTCPPCPAPELLGGPSVFLFPPKPKDTLMISRTPEVTCVVVDVSHEDPEVKFNWYVDGVEVHNAKTKPREEQYNSTYRVVSVLTVLHQDWLNGKEYKCKVSNKALPAPIEKTISKAKGQPREPQVYTLPPSREEMTKNQVSLTCLVKGFYPSDIAVEWESNGQPENNYKTTPPVLDSDGSFFLYSKLTVDKSRWQQGNVFSCSVMHEALHNHYTQKSLSLSPGK

SEQ ID NO: 4 - protein, 107 aa, synthetic construct [sequence omitted]

SEQ ID NO: 5 - protein, 5 aa, synthetic construct
DTYIH

SEQ ID NO: 6 - protein, 17 aa, synthetic construct
RIYPTNGYTRYADSVKG

SEQ ID NO: 7 - protein, 11 aa, synthetic construct
WGGDGFYAMDY

SEQ ID NO: 8 - protein, 11 aa, synthetic construct
RASQDVNTAVA

SEQ ID NO: 9 - protein, 7 aa, synthetic construct
SASFLYS

SEQ ID NO: 10 - protein, 9 aa, synthetic construct
QQHYTTPPT

SEQ ID NO: 11 - protein, 454 aa, synthetic construct
QVQLVQSGAEVKKPGSSVKVSCKASGGTFSDNDFSWVRQAPGQGLEWMGAIVAVFRTETYAQKFQDRVKITADISTRTTYMELSSLRSEDTAVYYCARRLMSAISGPGAPLLMWGQGTLVTVSSASTKGPSVCPLAPSSKSTSGGTAALGCLVKDYFPEPVTVSWNSGALTSGVHTFPAVLQSSGLYSLSSVVTVPSSSLGTQTYICNVNHKPSNTKVDKRVEPKSVDKTHTCPPCPAPEFEGGPSVFLFPPKPKDTLMISRTPEVTCVVVDVSHEDPEVKFNWYVDGVEVHNAKTKPREEQYNSTYRVVSVLTVLHQDWLNGKEYKCKVSNKALPASIEKTISKAKGQPREPQVYTLPPCREEMTKNQVSLWCLVKGFYPSDIAVEWESNGQPENNYKTTPPVLDSDGSFFLYSKLTVDKSRWQQGNVFSCSVMHEALHNHYTQKSLSLSPGK

SEQ ID NO: 12 - protein, 446 aa, synthetic construct
QVQLVQSGAEVKKPGASVKVSCKASGYTFTDYYIHWVRQATGQGLEWMGWMNPNSGNTGYAQKFQGRVTMTRDTSISTAYMELSSLRSEDTAVYYCARGQGYTHSWGQGTMVTVSSASTKGPSVFPLAPSSKSTSGGTAALGCLVKDYFPEPVTVSWNSGALTSGVHTFPAVLQSSGLYSLSSVVTVPSSSLGTQTYICNVNHKPSNTKVDKRVEPKSCDKTHTCPPCPAPEFEGGPSVFLFPPKPKDTLMISRTPEVTCVVVDVSHEDPEVKFNWYVDGVEVHNAKTKPREEQYNSTYRVVSVLTVLHQDWLNGKEYKCKVSNKALPASIEKTISKAKGQPREPQVCTLPPSREEMTKNQVSLSCAVKGFYPSDIAVEWESNGQPENNYKTTPPVLDSDGSFFLVSKLTVDKSRWQQGNVFSCSVMHEALHNHYTQKSLSLSPGK

SEQ ID NO: 13 - protein, 217 aa, synthetic construct
QSALTQPRSVSGSPGQSVTISCTGTSSDVGGYNYVSWYQQHPGKAPKLMIYDVSKRPSGVPDRFSGSKSGNTASLTISGLQAEDEADYYCSSYTSSDTLEIFGGGTKLTVLGQPKAAPSVTLFPPCSEELQANKATLVCLISDFYPGAVTVAWKADSSPVKAGVETTTPSKQSNNKYAASSYLSLTPEQWKSHRSYSCQVTHEGSTVEKTVAPTEVS

SEQ ID NO: 14 - protein, 214 aa, synthetic construct
DIQMTQSPSTLSASVGDRVTITCRASEGIYHWLAWYQQKPGKAPKLLIYKASSLASGVPSRFSGSGSGTEFTLTISSLQPDDFATYYCQQYSNYPPTFGGGTKLEIKRTVAAPSVFIFPPSDEQLKSGTASVVCLLNNFYPREAKVQWKVDNALQSGNSQESVTEQDSKDSTYSLSSTLTLSKADYEKHKVYACEVTHQGLSSPVTKSFNRGEC

SEQ ID NO: 15 - protein, 117 aa, synthetic construct
EVQLVQSGAEVKKPGSSVKVSCKASGYTFTNYWMHWVRQAPGQGLEWMGDIDPSHSETHYTQKFKDRVTITVDKSTSTAYMELSSLRSEDTAVYYCARGDLGRFDYWGQGTTVTVSS

SEQ ID NO: 16 - protein, 111 aa, synthetic construct
DIQMTQSPSSLSASVGDRVTITCRASESVSIHGTHLMHWYQQKPGKPPKLLIYAASNLESGVPSRFSGSGSETDFTFTISSLQPEDIATYYCQQSFEDPWTFGGGTKVEIK

SEQ ID NO: 17 - protein, 5 aa, synthetic construct
NYWMH

SEQ ID NO: 18 - protein, 17 aa, synthetic construct
DIDPSHSETHYTQKFKD

SEQ ID NO: 19 - protein, 8 aa, synthetic construct
GDLGRFDY

SEQ ID NO: 20 - protein, 15 aa, synthetic construct
RASESVSIHGTHLMH

SEQ ID NO: 21 - protein, 7 aa, synthetic construct
AASNLES

SEQ ID NO: 22 - protein, 9 aa, synthetic construct
QQSFEDPWT